European Patent Specification EP 3 473 254 B1, published January 24, 2024. Title: Selective inhibition of MALT1 protease by phenothiazine derivatives. Applicant: Helmholtz Zentrum München. The sequence listing filed with the application follows.

SEQUENCE LISTING (4 sequences)

SEQ ID NO: 1 - DNA, 21 bp, artificial sequence
  /note="Description of artificial sequence: mIL-2 forward primer"
gagtgccaattcgatgatgag

SEQ ID NO: 2 - DNA, 20 bp, artificial sequence
  /note="Description of artificial sequence: mIL-2 reverse primer"
agggcttgttgagatgatgc

SEQ ID NO: 3 - DNA, 20 bp, artificial sequence
  /note="Description of artificial sequence: mbeta-actin forward primer"
cctctatgccaacacagtgc

SEQ ID NO: 4 - DNA, 20 bp, artificial sequence
  /note="Description of artificial sequence: mbeta-actin reverse primer"
gtactcctgcttgctgatcc